European Patent Specification EP 3 635 014 B1, published September 27, 2023. Title: NOVEL HETERO-DIMERIC MULTI-SPECIFIC ANTIBODY FORMAT. Applicant: Numab Innovation AG. The sequence listing filed with the application follows.

SEQUENCE LISTING (30 sequences)

SEQ ID NO: 1 - protein, 264 aa, Artificial Sequence
  recombinant antibody sequence
DIQMTQSPSSLSASVGDRVTITCQASENIYSFLAWYQQKPGKAPKLLIYSASKLAAGVPSRFSGSGSGTDFTLTISSLQPEDFATYYCQQTNRYSNPDIYNVFGTGTKVTVLGGGGGSGGGGSGGGGSGGGGSEVQLVESGGGLVQPGGSLRLSCAASGIDFNSNYYMCWVRQAPGKGLEWIGCIYVGSHVNTYYANWAKGRFTISRDNSKNTVYLQMNSLRAEDTAVYYCATSGSSVLYFKFWGQGTLVTVSSGGGGSGGGGS

SEQ ID NO: 2 - protein, 114 aa, Artificial Sequence
  recombinant antibody sequence
DIQMTQSPSSLSASVGDRVTITCQSSQSVFSNNYLAWFQQKPGQSPKRLIYSASTLASGVPSRFSGSGSGTDFTLTISSLQPEDFATYYCLGSYACSSADCYVFGCGTKVTVLG

SEQ ID NO: 3 - protein, 119 aa, Artificial Sequence
  recombinant antibody sequence
EVQLVESGGGLVQPGGSLRLSCAASGFSLSSYDMSWVRQAPGKCLAWIGASYASGPTYYASWAKGRFTISRDNSKNTVYLQMNSLRAEDTATYFCARGGWTGTSHSNIWGQGTLVTVSS

SEQ ID NO: 4 - protein, 114 aa, Artificial Sequence
  recombinant antibody sequence
DIQMTQSPSSLSASVGDRVTITCQSSQSVFSNNYLAWFQQKPGQSPKRLIYSASTLASGVPSRFSGSGSGTDFTLTISSLQPEDFATYYCLGSYACSSADCYVFGTGTKVTVLG

SEQ ID NO: 5 - protein, 119 aa, Artificial Sequence
  recombinant antibody sequence
EVQLVESGGGLVQPGGSLRLSCAASGFSLSSYDMSWVRQAPGKGLAWIGASYASGPTYYASWAKGRFTISRDNSKNTVYLQMNSLRAEDTATYFCARGGWTGTSHSNIWGQGTLVTVSS

SEQ ID NO: 6 - protein, 114 aa, Artificial Sequence
  recombinant antibody sequence
DIQMTQSPSSLSASVGDRVTITCQSSESVYNNKRLSWYQQKPGKAPKLLIYTASSLASGVPSRFSGSGSGTDFTLTISSLQPEDFATYYCQGEFTCSNADCFTFGCGTKVTVLG

SEQ ID NO: 7 - protein, 123 aa, Artificial Sequence
  recombinant antibody sequence
EVQLVESGGGLVQPGGSLRLSCAASGFPLSSYAMIWVRQAPGKCLEWIGMILRAGNIYYASWVKGRFTISRDNSKNTVYLQMNSLRAEDTAVYYCARRHYNREGYPIGIGDLWGQGTLVTVSS

SEQ ID NO: 8 - protein, 114 aa, Artificial Sequence
  recombinant antibody sequence
DIQMTQSPSSLSASVGDRVTITCQSSESVYNNKRLSWYQQKPGKAPKLLIYTASSLASGVPSRFSGSGSGTDFTLTISSLQPEDFATYYCQGEFTCSNADCFTFGTGTKVTVLG

SEQ ID NO: 9 - protein, 123 aa, Artificial Sequence
  recombinant antibody sequence
EVQLVESGGGLVQPGGSLRLSCAASGFPLSSYAMIWVRQAPGKGLEWIGMILRAGNIYYASWVKGRFTISRDNSKNTVYLQMNSLRAEDTAVYYCARRHYNREGYPIGIGDLWGQGTLVTVSS

SEQ ID NO: 10 - protein, 112 aa, Artificial Sequence
  recombinant antibody sequence
DIQMTQSPSSLSASVGDRVTITCQSSESVYSNNQLSWYQQKPGQPPKLLIYDASDLASGVPSRFSGSGSGTDFTLTISSLQPEDFATYYCAGGFSSSSDTAFGGGTKLTVLG

SEQ ID NO: 11 - protein, 121 aa, Artificial Sequence
  recombinant antibody sequence
EVQLVESGGGLVQPGGSLRLSCAASGFSLSSNAMGWVRQAPGKGLEYIGIISVGGFTYYASWAKGRFTISRDNSKNTVYLQMNSLRAEDTATYFCARDRHGGDSSGAFYLWGQGTLVTVSS

SEQ ID NO: 12 - protein, 112 aa, Artificial Sequence
  recombinant antibody sequence
DIQMTQSPSSLSASVGDRVTITCQSSESVYSNNQLSWYQQKPGQPPKLLIYDASDLASGVPSRFSGSGSGTDFTLTISSLQPEDFATYYCAGGFSSSSDTAFGCGTKLTVLG

SEQ ID NO: 13 - protein, 121 aa, Artificial Sequence
  recombinant antibody sequence
EVQLVESGGGLVQPGGSLRLSCAASGFSLSSNAMGWVRQAPGKCLEYIGIISVGGFTYYASWAKGRFTISRDNSKNTVYLQMNSLRAEDTATYFCARDRHGGDSSGAFYLWGQGTLVTVSS

SEQ ID NO: 14 - protein, 110 aa, Artificial Sequence
  recombinant antibody sequence
DVVMTQSPSSLSASVGDRVTITCQASQIISSRSAWYQQKPGQPPKLLIYQASKLASGVPSRFSGSGSGTDFTLTISSLQPEDFATYYCQCTYIDSNFGAFGGGTKLTVLG

SEQ ID NO: 15 - protein, 121 aa, Artificial Sequence
  recombinant antibody sequence
EVQLVESGGGLVQPGGSLRLSCAASGFSFSSSYWICWVRQAPGKGLEWVGCVFTGDGTTYYASWAKGRFTISRDNSKNTVYLQMNSLRAEDTATYFCARPVSVYYYGMDLWGQGTLVTVSS

SEQ ID NO: 16 - protein, 14 aa, Artificial Sequence
  recombinant antibody sequence
EPEPEPEPEPEPEP

SEQ ID NO: 17 - protein, 14 aa, Artificial Sequence
  recombinant antibody sequence
KPKPKPKPKPKPKP

SEQ ID NO: 18 - protein, 11 aa, Artificial Sequence
  recombinant antibody sequence
SGGGGSGGGGS

SEQ ID NO: 19 - protein, 15 aa, Artificial Sequence
  recombinant antibody sequence
GGGGSGGGGSGGGGS

SEQ ID NO: 20 - protein, 12 aa, Artificial Sequence
  recombinant antibody sequence
AEAAAKEAAAKA

SEQ ID NO: 21 - protein, 258 aa, Artificial Sequence
  recombinant antibody sequence
DIQMTQSPSSLSASVGDRVTITCRASQDVNTAVAWYQQKPGKAPKLLIYSASFLYSGVPSRFSGSRSGTDFTLTISSLQPEDFATYYCQQHYTTPPTFGGGTKLTVLGGGGGSGGGGSGGGGSGGGGSEVQLVESGGGLVQPGGSLRLSCAASGFNIKDTYIHWVRQAPGKGLEWVARIYPTNGYTRYADSVKGRFTISADTSKNTAYLQMNSLRAEDTAVYYCSRWGGDGFYAMDYWGQGTLVTVSSGGGGSGGGGS

SEQ ID NO: 22 - protein, 504 aa, Artificial Sequence
  recombinant antibody sequence
DIQMTQSPSSLSASVGDRVTITCQASENIYSFLAWYQQKPGKAPKLLIYSASKLAAGVPSRFSGSGSGTDFTLTISSLQPEDFATYYCQQTNRYSNPDIYNVFGTGTKVTVLGGGGGSGGGGSGGGGSGGGGSEVQLVESGGGLVQPGGSLRLSCAASGIDFNSNYYMCWVRQAPGKGLEWIGCIYVGSHVNTYYANWAKGRFTISRDNSKNTVYLQMNSLRAEDTAVYYCATSGSSVLYFKFWGQGTLVTVSSGGGGSGGGGSDIQMTQSPSSLSASVGDRVTITCQSSQSVFSNNYLAWFQQKPGQSPKRLIYSASTLASGVPSRFSGSGSGTDFTLTISSLQPEDFATYYCLGSYACSSADCYVFGCGTKVTVLGEPEPEPEPEPEPEPDIQMTQSPSSLSASVGDRVTITCQSSESVYSNNQLSWYQQKPGQPPKLLIYDASDLASGVPSRFSGSGSGTDFTLTISSLQPEDFATYYCAGGFSSSSDTAFGGGTKLTVLG

SEQ ID NO: 23 - protein, 518 aa, Artificial Sequence
  recombinant antibody sequence
DIQMTQSPSSLSASVGDRVTITCQASENIYSFLAWYQQKPGKAPKLLIYSASKLAAGVPSRFSGSGSGTDFTLTISSLQPEDFATYYCQQTNRYSNPDIYNVFGTGTKVTVLGGGGGSGGGGSGGGGSGGGGSEVQLVESGGGLVQPGGSLRLSCAASGIDFNSNYYMCWVRQAPGKGLEWIGCIYVGSHVNTYYANWAKGRFTISRDNSKNTVYLQMNSLRAEDTAVYYCATSGSSVLYFKFWGQGTLVTVSSGGGGSGGGGSEVQLVESGGGLVQPGGSLRLSCAASGFSLSSNAMGWVRQAPGKGLEYIGIISVGGFTYYASWAKGRFTISRDNSKNTVYLQMNSLRAEDTATYFCARDRHGGDSSGAFYLWGQGTLVTVSSKPKPKPKPKPKPKPEVQLVESGGGLVQPGGSLRLSCAASGFSLSSYDMSWVRQAPGKCLAWIGASYASGPTYYASWAKGRFTISRDNSKNTVYLQMNSLRAEDTATYFCARGGWTGTSHSNIWGQGTLVTVSS

SEQ ID NO: 24 - protein, 11 aa, Artificial Sequence
  recombinant antibody sequence
FGTGTKVTVLG

SEQ ID NO: 25 - protein, 11 aa, Artificial Sequence
  recombinant antibody sequence
FGGGTKLTVLG

SEQ ID NO: 26 - protein, 11 aa, Artificial Sequence
  recombinant antibody sequence
FGGGTQLIILG

SEQ ID NO: 27 - protein, 11 aa, Artificial Sequence
  recombinant antibody sequence
FGEGTELTVLG

SEQ ID NO: 28 - protein, 11 aa, Artificial Sequence
  recombinant antibody sequence
FGSGTKVTVLG

SEQ ID NO: 29 - protein, 11 aa, Artificial Sequence
  recombinant antibody sequence
FGGGTQLTVLG

SEQ ID NO: 30 - protein, 11 aa, Artificial Sequence
  recombinant antibody sequence
FGGGTQLTALG